European Patent Application EP 4 206 318 A1, published July 5, 2023. Title: NME VARIANT SPECIES EXPRESSION AND SUPPRESSION. Applicant: Minerva Biotechnologies Corporation. Application EP 13823099.0, filed July 24, 2013. The sequence listing filed with the application follows.

SEQUENCE LISTING (51 sequences)

SEQ ID NO: 1 - protein, 1255 aa, synthetic construct
  REGION 1..1255: note = full-length MUC1 Receptor
MTPGTQSPFFLLLLLTVLTVVTGSGHASSTPGGEKETSATQRSSVPSSTEKNAVSMTSSVLSSHSPGSGSSTTQGQDVTLAPATEPASGSAATWGQDVTSVPVTRPALGSTTPPAHDVTSAPDNKPAPGSTAPPAHGVTSAPDTRPAPGSTAPPAHGVTSAPDTRPAPGSTAPPAHGVTSAPDTRPAPGSTAPPAHGVTSAPDTRPAPGSTAPPAHGVTSAPDTRPAPGSTAPPAHGVTSAPDTRPAPGSTAPPAHGVTSAPDTRPAPGSTAPPAHGVTSAPDTRPAPGSTAPPAHGVTSAPDTRPAPGSTAPPAHGVTSAPDTRPAPGSTAPPAHGVTSAPDTRPAPGSTAPPAHGVTSAPDTRPAPGSTAPPAHGVTSAPDTRPAPGSTAPPAHGVTSAPDTRPAPGSTAPPAHGVTSAPDTRPAPGSTAPPAHGVTSAPDTRPAPGSTAPPAHGVTSAPDTRPAPGSTAPPAHGVTSAPDTRPAPGSTAPPAHGVTSAPDTRPAPGSTAPPAHGVTSAPDTRPAPGSTAPPAHGVTSAPDTRPAPGSTAPPAHGVTSAPDTRPAPGSTAPPAHGVTSAPDTRPAPGSTAPPAHGVTSAPDTRPAPGSTAPPAHGVTSAPDTRPAPGSTAPPAHGVTSAPDTRPAPGSTAPPAHGVTSAPDTRPAPGSTAPPAHGVTSAPDTRPAPGSTAPPAHGVTSAPDTRPAPGSTAPPAHGVTSAPDTRPAPGSTAPPAHGVTSAPDTRPAPGSTAPPAHGVTSAPDTRPAPGSTAPPAHGVTSAPDTRPAPGSTAPPAHGVTSAPDTRPAPGSTAPPAHGVTSAPDTRPAPGSTAPPAHGVTSAPDTRPAPGSTAPPAHGVTSAPDTRPAPGSTAPPAHGVTSAPDTRPAPGSTAPPAHGVTSAPDTRPAPGSTAPPAHGVTSAPDTRPAPGSTAPPAHGVTSAPDNRPALGSTAPPVHNVTSASGSASGSASTLVHNGTSARATTTPASKSTPFSIPSHHSDTPTTLASHSTKTDASSTHHSSVPPLTSSNHSTSPQLSTGVSFFFLSFHISNLQFNSSLEDPSTDYYQELQRDISEMFLQIYKQGGFLGLSNIKFRPGSVVVQLTLAFREGTINVHDVETQFNQYKTEAASRYNLTISDVSVSDVPFPFSAQSGAGVPGWGIALLVLVCVLVALAIVYLIALAVCQCRRKNYGQLDIFPARDTYHPMSEYPTYHTHGRYVPPSSTDRSPYEKVSAGNGGSSLSYTNPAVAAASANL

SEQ ID NO: 2 - protein, 19 aa, synthetic construct
  REGION 1..19: note = N-terminal MUC-1 signaling sequence
MTPGTQSPFFLLLLLTVLT

SEQ ID NO: 3 - protein, 23 aa, synthetic construct
  REGION 1..23: note = N-terminal MUC-1 signaling sequence
MTPGTQSPFFLLLLLTVLTVVTA

SEQ ID NO: 4 - protein, 23 aa, synthetic construct
  REGION 1..23: note = N-terminal MUC-1 signaling sequence
MTPGTQSPFFLLLLLTVLTVVTG

SEQ ID NO: 5 - protein, 146 aa, synthetic construct
  REGION 1..146: note = truncated MUC1 receptor isoform
GTINVHDVETQFNQYKTEAASRYNLTISDVSVSDVPFPFSAQSGAGVPGWGIALLVLVCVLVALAIVYLIALAVCQCRRKNYGQLDIFPARDTYHPMSEYPTYHTHGRYVPPSSTDRSPYEKVSAGNGGSSLSYTNPAVAAASANL

SEQ ID NO: 6 - protein, 45 aa, synthetic construct
  REGION 1..45: note = Native Primary Sequence of the MUC1 Growth Factor Receptor
GTINVHDVETQFNQYKTEAASRYNLTISDVSVSDVPFPFSAQSGA

SEQ ID NO: 7 - protein, 44 aa, synthetic construct
  REGION 1..44: note = Native Primary Sequence of the MUC1 Growth Factor Receptor
TINVHDVETQFNQYKTEAASRYNLTISDVSVSDVPFPFSAQSGA

SEQ ID NO: 8 - protein, 45 aa, synthetic construct
  REGION 1..45: note = "SPY" functional variant of the native Primary Sequence of theMUC1 Growth Factor Receptor
GTINVHDVETQFNQYKTEAASPYNLTISDVSVSDVPFPFSAQSGA

SEQ ID NO: 9 - protein, 44 aa, synthetic construct
  REGION 1..44: note = "SPY" functional variant of the native Primary Sequence of theMUC1 Growth Factor Receptor
TINVHDVETQFNQYKTEAASPYNLTISDVSVSDVPFPFSAQSGA

SEQ ID NO: 10 - DNA, 216 bp, synthetic construct
  misc_feature 1..216: note = MUC1 cytoplasmic domain nucleotide sequence
  source 1..216: mol_type = other DNA
tgtcagtgccgccgaaagaactacgggcagctggacatctttccagcccgggatacctaccatcctatgagcgagtaccccacctaccacacccatgggcgctatgtgccccctagcagtaccgatcgtagcccctatgagaaggtttctgcaggtaacggtggcagcagcctctcttacacaaacccagcagtggcagccgcttctgccaacttg

SEQ ID NO: 11 - protein, 72 aa, synthetic construct
  REGION 1..72: note = MUC1 cytoplasmic domain amino acid sequence
CQCRRKNYGQLDIFPARDTYHPMSEYPTYHTHGRYVPPSSTDRSPYEKVSAGNGGSSLSYTNPAVAAASANL

SEQ ID NO: 12 - DNA, 459 bp, synthetic construct
  misc_feature 1..459: note = Human NM23 H1
  source 1..459: mol_type = other DNA
atggccaactgtgagcgtaccttcattgcgatcaaaccagatggggtccagcggggtcttgtgggagagattatcaagcgttttgagcagaaaggattccgccttgttggtctgaaattcatgcaagcttccgaagatcttctcaaggaacactacgttgacctgaaggaccgtccattctttgccggcctggtgaaatacatgcactcagggccggtagttgccatggtctgggaggggctgaatgtggtgaagacgggccgagtcatgctcggggagaccaaccctgcagactccaagcctgggaccatccgtggagacttctgcatacaagttggcaggaacattatacatggcagtgattctgtggagagtgcagagaaggagatcggcttgtggtttcaccctgaggaactggtagattacacgagctgtgctcagaactggatctatgaatga

SEQ ID NO: 13 - protein, 152 aa, synthetic construct
  REGION 1..152: note = Human NM23 H1
MANCERTFIAIKPDGVQRGLVGEIIKRFEQKGFRLVGLKFMQASEDLLKEHYVDLKDRPFFAGLVKYMHSGPVVAMVWEGLNVVKTGRVMLGETNPADSKPGTIRGDFCIQVGRNIIHGSDSVESAEKEIGLWFHPEELVDYTSCAQNWIYE

SEQ ID NO: 14 - DNA, 459 bp, synthetic construct
  misc_feature 1..459: note = Mouse NM23 H1
  source 1..459: mol_type = other DNA
atggccaacagtgagcgcaccttcattgccatcaagcctgatggggtccagcgggggctggtgggcgagatcatcaagcggttcgagcagaaggggttccgccttgttggtctgaagtttctgcaggcttcagaggaccttctcaaggagcactacactgacctgaaggaccgccccttctttactggcctggtgaaatacatgcactcaggaccagtggttgctatggtctgggagggtctgaatgtggtgaagacaggccgcgtgatgcttggagagaccaaccccgcagactctaagcctgggaccatacgaggagacttctgcatccaagttggcaggaacatcattcatggcagcgattctgtaaagagcgcagagaaggagatcagcttgtggtttcagcctgaggagctggtggagtacaagagctgtgcgcagaactggatctatgagtga

SEQ ID NO: 15 - protein, 152 aa, synthetic construct
  REGION 1..152: note = Mouse NM23 H1
MANSERTFIAIKPDGVQRGLVGEIIKRFEQKGFRLVGLKFLQASEDLLKEHYTDLKDRPFFTGLVKYMHSGPVVAMVWEGLNVVKTGRVMLGETNPADSKPGTIRGDFCIQVGRNIIHGSDSVKSAEKEISLWFQPEELVEYKSCAQNWIYE

SEQ ID NO: 16 - DNA, 459 bp, synthetic construct
  misc_feature 1..459: note = Human NM23 H2
  source 1..459: mol_type = other DNA
atggccaacctggagcgcaccttcatcgccatcaagccggacggcgtgcagcgcggcctggtgggcgagatcatcaagcgcttcgagcagaagggattccgcctcgtggccatgaagttcctccgggcctctgaagaacacctgaagcagcactacattgacctgaaagaccgaccattcttccctgggctggtgaagtacatgaactcagggccggttgtggccatggtctgggaggggctgaacgtggtgaagacaggccgagtgatgcttggggagaccaatccagcagattcaaagccaggcaccattcgtggggacttctgcattcaggttggcaggaacatcattcatggcagtgattcagtaaaaagtgctgaaaaagaaatcagcctatggtttaagcctgaagaactggttgactacaagtcttgtgctcatgactgggtctatgaataa

SEQ ID NO: 17 - protein, 152 aa, synthetic construct
  REGION 1..152: note = Human NM23 H2
MANLERTFIAIKPDGVQRGLVGEIIKRFEQKGFRLVAMKFLRASEEHLKQHYIDLKDRPFFPGLVKYMNSGPVVAMVWEGLNVVKTGRVMLGETNPADSKPGTIRGDFCIQVGRNIIHGSDSVKSAEKEISLWFKPEELVDYKSCAHDWVYE

SEQ ID NO: 18 - DNA, 459 bp, synthetic construct
  misc_feature 1..459: note = Mouse NM23 H2
  source 1..459: mol_type = other DNA
atggccaacctcgagcgtaccttcattgccatcaagccagatggcgtgcagcgcggcctggtgggcgagatcatcaaacggttcgagcagaaggggttccgcctggtggccatgaagttccttcgggcctctgaagaacacctgaagcagcattacatcgacctgaaagaccgtcctttcttcccggggctggtgaagtacatgaactcggggcccgtggtggccatggtctgggaggggctcaatgtggtgaaaacgggccgagtgatgctgggggagaccaatccagctgattcaaaaccaggcaccatccgtggggatttctgcattcaagttggcaggaacatcattcatggcagtgattcagtggagagtgctgagaaagagatccatctgtggtttaagcccgaagaactgatcgactacaagtcttgtgcccatgactgggtgtacgagtag

SEQ ID NO: 19 - protein, 152 aa, synthetic construct
  REGION 1..152: note = Mouse NM23 H2
MANLERTFIAIKPDGVQRGLVGEIIKRFEQKGFRLVAMKFLRASEEHLKQHYIDLKDRPFFPGLVKYMNSGPVVAMVWEGLNVVKTGRVMLGETNPADSKPGTIRGDFCIQVGRNIIHGSDSVESAEKEIHLWFKPEELIDYKSCAHDWVYE

SEQ ID NO: 20 - DNA, 570 bp, synthetic construct
  misc_feature 1..570: note = Mouse NME6
  source 1..570: mol_type = other DNA
atgacctccatcttgcgaagtccccaagctcttcagctcacactagccctgatcaagcctgatgcagttgcccacccactgatcctggaggctgttcatcagcagattctgagcaacaagttcctcattgtacgaacgagggaactgcagtggaagctggaggactgccggaggttttaccgagagcatgaagggcgttttttctatcagcggctggtggagttcatgacaagtgggccaatccgagcctatatccttgcccacaaagatgccatccaactttggaggacactgatgggacccaccagagtatttcgagcacgctatatagccccagattcaattcgtggaagtttgggcctcactgacacccgaaatactacccatggctcagactccgtggtttccgccagcagagagattgcagccttcttccctgacttcagtgaacagcgctggtatgaggaggaggaaccccagctgcggtgtggtcctgtgcactacagtccagaggaaggtatccactgtgcagctgaaacaggaggccacaaacaacctaacaaaacctag

SEQ ID NO: 21 - protein, 189 aa, synthetic construct
  REGION 1..189: note = Mouse NME6
MTSILRSPQALQLTLALIKPDAVAHPLILEAVHQQILSNKFLIVRTRELQWKLEDCRRFYREHEGRFFYQRLVEFMTSGPIRAYILAHKDAIQLWRTLMGPTRVFRARYIAPDSIRGSLGLTDTRNTTHGSDSVVSASREIAAFFPDFSEQRWYEEEEPQLRCGPVHYSPEEGIHCAAETGGHKQPNKT

SEQ ID NO: 22 - DNA, 585 bp, synthetic construct
  misc_feature 1..585: note = Human NME6
  source 1..585: mol_type = other DNA
atgacccagaatctggggagtgagatggcctcaatcttgcgaagccctcaggctctccagctcactctagccctgatcaagcctgacgcagtcgcccatccactgattctggaggctgttcatcagcagattctaagcaacaagttcctgattgtacgaatgagagaactactgtggagaaaggaagattgccagaggttttaccgagagcatgaagggcgttttttctatcagaggctggtggagttcatggccagcgggccaatccgagcctacatccttgcccacaaggatgccatccagctctggaggacgctcatgggacccaccagagtgttccgagcacgccatgtggccccagattctatccgtgggagtttcggcctcactgacacccgcaacaccacccatggttcggactctgtggtttcagccagcagagagattgcagccttcttccctgacttcagtgaacagcgctggtatgaggaggaagagccccagttgcgctgtggccctgtgtgctatagcccagagggaggtgtccactatgtagctggaacaggaggcctaggaccagcctga

SEQ ID NO: 23 - protein, 194 aa, synthetic construct
  REGION 1..194: note = Human NME6
MTQNLGSEMASILRSPQALQLTLALIKPDAVAHPLILEAVHQQILSNKFLIVRMRELLWRKEDCQRFYREHEGRFFYQRLVEFMASGPIRAYILAHKDAIQLWRTLMGPTRVFRARHVAPDSIRGSFGLTDTRNTTHGSDSVVSASREIAAFFPDFSEQRWYEEEEPQLRCGPVCYSPEGGVHYVAGTGGLGPA

SEQ ID NO: 24 - DNA, 525 bp, synthetic construct
  misc_feature 1..525: note = Human NME6 1
  source 1..525: mol_type = other DNA
atgacccagaatctggggagtgagatggcctcaatcttgcgaagccctcaggctctccagctcactctagccctgatcaagcctgacgcagtcgcccatccactgattctggaggctgttcatcagcagattctaagcaacaagttcctgattgtacgaatgagagaactactgtggagaaaggaagattgccagaggttttaccgagagcatgaagggcgttttttctatcagaggctggtggagttcatggccagcgggccaatccgagcctacatccttgcccacaaggatgccatccagctctggaggacgctcatgggacccaccagagtgttccgagcacgccatgtggccccagattctatccgtgggagtttcggcctcactgacacccgcaacaccacccatggttcggactctgtggtttcagccagcagagagattgcagccttcttccctgacttcagtgaacagcgctggtatgaggaggaagagccccagttgcgctgtggccctgtgtga

SEQ ID NO: 25 - protein, 174 aa, synthetic construct
  REGION 1..174: note = Human NME6 1
MTQNLGSEMASILRSPQALQLTLALIKPDAVAHPLILEAVHQQILSNKFLIVRMRELLWRKEDCQRFYREHEGRFFYQRLVEFMASGPIRAYILAHKDAIQLWRTLMGPTRVFRARHVAPDSIRGSFGLTDTRNTTHGSDSVVSASREIAAFFPDFSEQRWYEEEEPQLRCGPV

SEQ ID NO: 26 - DNA, 468 bp, synthetic construct
  misc_feature 1..468: note = Human NME6 2
  source 1..468: mol_type = other DNA
atgctcactctagccctgatcaagcctgacgcagtcgcccatccactgattctggaggctgttcatcagcagattctaagcaacaagttcctgattgtacgaatgagagaactactgtggagaaaggaagattgccagaggttttaccgagagcatgaagggcgttttttctatcagaggctggtggagttcatggccagcgggccaatccgagcctacatccttgcccacaaggatgccatccagctctggaggacgctcatgggacccaccagagtgttccgagcacgccatgtggccccagattctatccgtgggagtttcggcctcactgacacccgcaacaccacccatggttcggactctgtggtttcagccagcagagagattgcagccttcttccctgacttcagtgaacagcgctggtatgaggaggaagagccccagttgcgctgtggccctgtgtga

SEQ ID NO: 27 - protein, 155 aa, synthetic construct
  REGION 1..155: note = Human NME6 2
MLTLALIKPDAVAHPLILEAVHQQILSNKFLIVRMRELLWRKEDCQRFYREHEGRFFYQRLVEFMASGPIRAYILAHKDAIQLWRTLMGPTRVFRARHVAPDSIRGSFGLTDTRNTTHGSDSVVSASREIAAFFPDFSEQRWYEEEEPQLRCGPV

SEQ ID NO: 28 - DNA, 528 bp, synthetic construct
  misc_feature 1..528: note = Human NME6 3
  source 1..528: mol_type = other DNA
atgctcactctagccctgatcaagcctgacgcagtcgcccatccactgattctggaggctgttcatcagcagattctaagcaacaagttcctgattgtacgaatgagagaactactgtggagaaaggaagattgccagaggttttaccgagagcatgaagggcgttttttctatcagaggctggtggagttcatggccagcgggccaatccgagcctacatccttgcccacaaggatgccatccagctctggaggacgctcatgggacccaccagagtgttccgagcacgccatgtggccccagattctatccgtgggagtttcggcctcactgacacccgcaacaccacccatggttcggactctgtggtttcagccagcagagagattgcagccttcttccctgacttcagtgaacagcgctggtatgaggaggaagagccccagttgcgctgtggccctgtgtgctatagcccagagggaggtgtccactatgtagctggaacaggaggcctaggaccagcctga

SEQ ID NO: 29 - protein, 175 aa, synthetic construct
  REGION 1..175: note = Human NME6 3
MLTLALIKPDAVAHPLILEAVHQQILSNKFLIVRMRELLWRKEDCQRFYREHEGRFFYQRLVEFMASGPIRAYILAHKDAIQLWRTLMGPTRVFRARHVAPDSIRGSFGLTDTRNTTHGSDSVVSASREIAAFFPDFSEQRWYEEEEPQLRCGPVCYSPEGGVHYVAGTGGLGPA

SEQ ID NO: 30 - DNA, 1131 bp, synthetic construct
  misc_feature 1..1131: note = Human NM23-H7-1
  source 1..1131: mol_type = other DNA
atgaatcatagtgaaagattcgttttcattgcagagtggtatgatccaaatgcttcacttcttcgacgttatgagcttttattttacccaggggatggatctgttgaaatgcatgatgtaaagaatcatcgcacctttttaaagcggaccaaatatgataacctgcacttggaagatttatttataggcaacaaagtgaatgtcttttctcgacaactggtattaattgactatggggatcaatatacagctcgccagctgggcagtaggaaagaaaaaacgctagccctaattaaaccagatgcaatatcaaaggctggagaaataattgaaataataaacaaagctggatttactataaccaaactcaaaatgatgatgctttcaaggaaagaagcattggattttcatgtagatcaccagtcaagaccctttttcaatgagctgatccagtttattacaactggtcctattattgccatggagattttaagagatgatgctatatgtgaatggaaaagactgctgggacctgcaaactctggagtggcacgcacagatgcttctgaaagcattagagccctctttggaacagatggcataagaaatgcagcgcatggccctgattcttttgcttctgcggccagagaaatggagttgttttttccttcaagtggaggttgtgggccggcaaacactgctaaatttactaattgtacctgttgcattgttaaaccccatgctgtcagtgaaggactgttgggaaagatcctgatggctatccgagatgcaggttttgaaatctcagctatgcagatgttcaatatggatcgggttaatgttgaggaattctatgaagtttataaaggagtagtgaccgaatatcatgacatggtgacagaaatgtattctggcccttgtgtagcaatggagattcaacagaataatgctacaaagacatttcgagaattttgtggacctgctgatcctgaaattgcccggcatttacgccctggaactctcagagcaatctttggtaaaactaagatccagaatgctgttcactgtactgatctgccagaggatggcctattagaggttcaatacttcttcaagatcttggataattag

SEQ ID NO: 31 - protein, 376 aa, synthetic construct
  REGION 1..376: note = Human NM23-H7-1
MNHSERFVFIAEWYDPNASLLRRYELLFYPGDGSVEMHDVKNHRTFLKRTKYDNLHLEDLFIGNKVNVFSRQLVLIDYGDQYTARQLGSRKEKTLALIKPDAISKAGEIIEIINKAGFTITKLKMMMLSRKEALDFHVDHQSRPFFNELIQFITTGPIIAMEILRDDAICEWKRLLGPANSGVARTDASESIRALFGTDGIRNAAHGPDSFASAAREMELFFPSSGGCGPANTAKFTNCTCCIVKPHAVSEGLLGKILMAIRDAGFEISAMQMFNMDRVNVEEFYEVYKGVVTEYHDMVTEMYSGPCVAMEIQQNNATKTFREFCGPADPEIARHLRPGTLRAIFGKTKIQNAVHCTDLPEDGLLEVQYFFKILDN

SEQ ID NO: 32 - DNA, 1131 bp, synthetic construct
  misc_feature 1..1131: note = Human NM23-H7-1 sequence optimized for E. coli expression
  source 1..1131: mol_type = other DNA
atgaatcactccgaacgctttgtttttatcgccgaatggtatgacccgaatgcttccctgctgcgccgctacgaactgctgttttatccgggcgatggtagcgtggaaatgcatgacgttaaaaatcaccgtacctttctgaaacgcacgaaatatgataatctgcatctggaagacctgtttattggcaacaaagtcaatgtgttctctcgtcagctggtgctgatcgattatggcgaccagtacaccgcgcgtcaactgggtagtcgcaaagaaaaaacgctggccctgattaaaccggatgcaatctccaaagctggcgaaattatcgaaattatcaacaaagcgggtttcaccatcacgaaactgaaaatgatgatgctgagccgtaaagaagccctggattttcatgtcgaccaccagtctcgcccgtttttcaatgaactgattcaattcatcaccacgggtccgattatcgcaatggaaattctgcgtgatgacgctatctgcgaatggaaacgcctgctgggcccggcaaactcaggtgttgcgcgtaccgatgccagtgaatccattcgcgctctgtttggcaccgatggtatccgtaatgcagcacatggtccggactcattcgcatcggcagctcgtgaaatggaactgtttttcccgagctctggcggttgcggtccggcaaacaccgccaaatttaccaattgtacgtgctgtattgtcaaaccgcacgcagtgtcagaaggcctgctgggtaaaattctgatggcaatccgtgatgctggctttgaaatctcggccatgcagatgttcaacatggaccgcgttaacgtcgaagaattctacgaagtttacaaaggcgtggttaccgaatatcacgatatggttacggaaatgtactccggtccgtgcgtcgcgatggaaattcagcaaaacaatgccaccaaaacgtttcgtgaattctgtggtccggcagatccggaaatcgcacgtcatctgcgtccgggtaccctgcgcgcaatttttggtaaaacgaaaatccagaacgctgtgcactgtaccgatctgccggaagacggtctgctggaagttcaatactttttcaaaattctggataattag

SEQ ID NO: 33 - protein, 376 aa, synthetic construct; identical to SEQ ID NO: 31
  REGION 1..376: note = Human NM23-H7-1 sequence optimized for E. coli expression

SEQ ID NO: 34 - DNA, 1023 bp, synthetic construct
  misc_feature 1..1023: note = Human NM23-H7-2
  source 1..1023: mol_type = other DNA
atgcatgatgtaaagaatcatcgcacctttttaaagcggaccaaatatgataacctgcacttggaagatttatttataggcaacaaagtgaatgtcttttctcgacaactggtattaattgactatggggatcaatatacagctcgccagctgggcagtaggaaagaaaaaacgctagccctaattaaaccagatgcaatatcaaaggctggagaaataattgaaataataaacaaagctggatttactataaccaaactcaaaatgatgatgctttcaaggaaagaagcattggattttcatgtagatcaccagtcaagaccctttttcaatgagctgatccagtttattacaactggtcctattattgccatggagattttaagagatgatgctatatgtgaatggaaaagactgctgggacctgcaaactctggagtggcacgcacagatgcttctgaaagcattagagccctctttggaacagatggcataagaaatgcagcgcatggccctgattcttttgcttctgcggccagagaaatggagttgttttttccttcaagtggaggttgtgggccggcaaacactgctaaatttactaattgtacctgttgcattgttaaaccccatgctgtcagtgaaggactgttgggaaagatcctgatggctatccgagatgcaggttttgaaatctcagctatgcagatgttcaatatggatcgggttaatgttgaggaattctatgaagtttataaaggagtagtgaccgaatatcatgacatggtgacagaaatgtattctggcccttgtgtagcaatggagattcaacagaataatgctacaaagacatttcgagaattttgtggacctgctgatcctgaaattgcccggcatttacgccctggaactctcagagcaatctttggtaaaactaagatccagaatgctgttcactgtactgatctgccagaggatggcctattagaggttcaatacttcttcaagatcttggataattga

SEQ ID NO: 35 - protein, 340 aa, synthetic construct
  REGION 1..340: note = Human NM23-H7-2
MHDVKNHRTFLKRTKYDNLHLEDLFIGNKVNVFSRQLVLIDYGDQYTARQLGSRKEKTLALIKPDAISKAGEIIEIINKAGFTITKLKMMMLSRKEALDFHVDHQSRPFFNELIQFITTGPIIAMEILRDDAICEWKRLLGPANSGVARTDASESIRALFGTDGIRNAAHGPDSFASAAREMELFFPSSGGCGPANTAKFTNCTCCIVKPHAVSEGLLGKILMAIRDAGFEISAMQMFNMDRVNVEEFYEVYKGVVTEYHDMVTEMYSGPCVAMEIQQNNATKTFREFCGPADPEIARHLRPGTLRAIFGKTKIQNAVHCTDLPEDGLLEVQYFFKILDN

SEQ ID NO: 36 - DNA, 1188 bp, synthetic construct
  misc_feature 1..1188: note = Mouse NM23-H7-1
  source 1..1188: mol_type = other DNA
atgagagcctgtcagcagggaagaagttccagtttggtttctccatatatggcacccaagaatcagagcgagagattcgctttcattgcagagtggtatgatccaaatgcttcattgctccgacgctatgagctgctgttttaccccacagacggatctgttgaaatgcatgatgtaaagaatcgtcgcaccttcttaaagcggaccaagtatgaggacctgcgcctggaagatctatttataggcaacaaagtcaatgtgttttctcgacagctggtgttgattgactatggggaccaatacacagcccgccagctgggcagcaggaaagagaaaactttagccctgatcaaaccagatgcagtgtcaaaggccggagaaatcattgagatgataaacaaaagtggatttactataaccaaactccgaatgatgactctgacaaggaaagaagcagcggactttcatgtagaccatcactcaagacctttttataacgaactgatccagtttatcacaagtgggcctgttattgccatggagatcttaagagatgacgcgatctgtgagtggaaaaggttgcttggacccgcaaactctgggctatcacggacagatgcccccggaagcatccgagccctctttgggacagatggcgtgagaaatgcagctcacggccctgatacttttgcatctgctgccagagaaatggaattgttttttccttcaagtggaggctgtgggccagcgaacactgctaaatttaccaattgcacctgttgcatcattaagcctcatgctatcagtgaaggaatgttgggaaagattttaatagctattcgggatgcatgctttggaatgtcagcgatacagatgttcaatttggatcgggctaatgttgaagaattctatgaagtctataaaggtgtagtgtctgagtataatgatatggtgacagagctgtgctccggcccttgcgtagcaatagagatccaacagagcaaccctacaaagacatttcgagaattctgcggacctgctgatcctgaaatcgcccggcatttacgacctgagaccctcagggcaatttttggtaaaactaaggttcaaaatgctgttcattgcacggatctgccggaggatgggctcctggaggtccagtatttcttcaagatcttggataattag

SEQ ID NO: 37 - protein, 395 aa, synthetic construct
  REGION 1..395: note = Mouse NM23-H7-1
MRACQQGRSSSLVSPYMAPKNQSERFAFIAEWYDPNASLLRRYELLFYPTDGSVEMHDVKNRRTFLKRTKYEDLRLEDLFIGNKVNVFSRQLVLIDYGDQYTARQLGSRKEKTLALIKPDAVSKAGEIIEMINKSGFTITKLRMMTLTRKEAADFHVDHHSRPFYNELIQFITSGPVIAMEILRDDAICEWKRLLGPANSGLSRTDAPGSIRALFGTDGVRNAAHGPDTFASAAREMELFFPSSGGCGPANTAKFTNCTCCIIKPHAISEGMLGKILIAIRDACFGMSAIQMFNLDRANVEEFYEVYKGVVSEYNDMVTELCSGPCVAIEIQQSNPTKTFREFCGPADPEIARHLRPETLRAIFGKTKVQNAVHCTDLPEDGLLEVQYFFKILDN

SEQ ID NO: 38 - DNA, 834 bp, synthetic construct
  misc_feature 1..834: note = Mouse NM23-H7-2
  source 1..834: mol_type = other DNA
atgagagcctgtcagcagggaagaagttccagtttggtttctccatatatggcacccaagaatcagagcgagagattcgctttcattgcagagtggtatgatccaaatgcttcattgctccgacgctatgagctgctgttttaccccacagacggatctgttgaaatgcatgatgtaaagaatcgtcgcaccttcttaaagcggaccaagtatgaggacctgcgcctggaagatctatttataggcaacaaagtcaatgtgttttctcgacagctggtgttgattgactatggggaccaatacacagcccgccagctgggcagcaggaaagagaaaactttagccctgatcaaaccagatgcagtgtcaaaggccggagaaatcattgagatgataaacaaaagtggatttactataaccaaactccgaatgatgactctgacaaggaaagaagcagcggactttcatgtagaccatcactcaagacctttttataacgaactgatccagtttatcacaagtgggcctgttattgccatggagatcttaagagatgacgcgatctgtgagtggaaaaggttgcttggacccgcaaactctgggctatcacggacagatgcccccggaagcatccgagccctctttgggacagatggcgtgagaaatgcagctcacggccctgatacttttgcatctgctgccagagaaatggaattgttttttccttcaagtggaggctgtgggccagcgaacactgctaaatttaccaattgcacctgttgcatcattaagcctcatgctatcagtgaagatttatttattcattatatgtaa

SEQ ID NO: 39 - protein, 277 aa, synthetic construct
  REGION 1..277: note = Mouse NM23-H7-2
MRACQQGRSSSLVSPYMAPKNQSERFAFIAEWYDPNASLLRRYELLFYPTDGSVEMHDVKNRRTFLKRTKYEDLRLEDLFIGNKVNVFSRQLVLIDYGDQYTARQLGSRKEKTLALIKPDAVSKAGEIIEMINKSGFTITKLRMMTLTRKEAADFHVDHHSRPFYNELIQFITSGPVIAMEILRDDAICEWKRLLGPANSGLSRTDAPGSIRALFGTDGVRNAAHGPDTFASAAREMELFFPSSGGCGPANTAKFTNCTCCIIKPHAISEDLFIHYM

SEQ ID NO: 40 - DNA, 1761 bp, synthetic construct
  misc_feature 1..1761: note = Mouse NME8 variant1
  source 1..1761: mol_type = other DNA
atggcaagcaaaaagcgtgaagtccagctacagtcagtcgtcaatagtcagaacttgtgggatgagatgttgctgaacaaaggcttaacagtgattgatgtttaccaagcctggtgtggaccttgcaaagccgtgcaaagtttattcagaaaactaaaaaatgaactgaacgaagatgagattcttcacttcgtcgttgctgaagctgacaacattgtgactctccagccatttagagataaatgtgagcccgtgtttctctttagtcttaatggtaaaatcattgcaaagattcagggtgcaaatgctccacttatcaatagaaaagtcattaccttgatagatgaagagaggaaaattgtagcaggtgaaatggatcgtcctcagtatgttgaaattccactagtagatgcaatcgatgaagaatatggggaagtacagtatgaaagtgctgcggaagtttacaatatggcaattatcaaacctgatgctgtactcatgagaaaaaatatagaagttagggaaaaaatagccaaagaaggatttgttatagaaatacaagaaaacctgattctccctgaagaggtagtgagggaattctacactcatatagcagaccagcctgactttgaagagtttgtcgtttctatgacaaatggcctcagctgtgtgctcattgtatctcaagaagactccgaggttattcaggaagaaactctcccgcagactgatacagaagaagaacctggcgttttggaagagcctcacgttaggtttgcacctgtgatgataaagaagaaacgggacagtttgcaagagtatatggaccgacagcatatgtctgattactgcgatgtcgaggacgatgcggttaaggtctctaagctcattgacatattattccctgattttaaaactatgaaaagcacgaatgtacaaacgacgctagcattactgcatccagacatctgtgaggaagagaaagatgacgtgttgaacgttattcacaatgaagggttcaccatactgatgcagaggcaaatcgtattatcagaggaagaagcaagaacagtgtgcaagatccatgaaaacgaagagtattttgataatcttatagggcacatgaccagtaatcactcttatgtccttgctctacggagggaaaatggtgtggaatattggaaaacattaattgggccaaaaacgattgaggaagcttatgcatctcatccacagagtttatgtgtacagtttgcttcagggaattttcctaccaaccagttctacgggagcagttcaaaagcagcagctgagaaggaaatagcgcatttcttccctccccagagcacacttgcattgatcaagcctcatgtgacacacaaagaaagaatggagatcctgaagaccattaaagaggcaggatttgagctgaccctgatgaaggaaatgcacctgactccagagcatgcaaacaaaatttatttcaaaataacaggaaaagatttttataaaaatgtattggaagtcttatctttgggcatgtcgctagtcatggttttgaccaagtggaatgctgttgcagaatggaggcgaatggttggcccagtagacccagaagaagcaaaactgctctccccagaatccctccgagccaaatatggactagacattttgagaaatgctgtccatggggcgtctaacttttctgaagcatcagaaatcattagtaatgtgttcacagagggtaatcctgagaactag

SEQ ID NO: 41 - protein, 586 aa, synthetic construct
  REGION 1..586: note = Mouse NME8 variant1
MASKKREVQLQSVVNSQNLWDEMLLNKGLTVIDVYQAWCGPCKAVQSLFRKLKNELNEDEILHFVVAEADNIVTLQPFRDKCEPVFLFSLNGKIIAKIQGANAPLINRKVITLIDEERKIVAGEMDRPQYVEIPLVDAIDEEYGEVQYESAAEVYNMAIIKPDAVLMRKNIEVREKIAKEGFVIEIQENLILPEEVVREFYTHIADQPDFEEFVVSMTNGLSCVLIVSQEDSEVIQEETLPQTDTEEEPGVLEEPHVRFAPVMIKKKRDSLQEYMDRQHMSDYCDVEDDAVKVSKLIDILFPDFKTMKSTNVQTTLALLHPDICEEEKDDVLNVIHNEGFTILMQRQIVLSEEEARTVCKIHENEEYFDNLIGHMTSNHSYVLALRRENGVEYWKTLIGPKTIEEAYASHPQSLCVQFASGNFPTNQFYGSSSKAAAEKEIAHFFPPQSTLALIKPHVTHKERMEILKTIKEAGFELTLMKEMHLTPEHANKIYFKITGKDFYKNVLEVLSLGMSLVMVLTKWNAVAEWRRMVGPVDPEEAKLLSPESLRAKYGLDILRNAVHGASNFSEASEIISNVFTEGNPEN

SEQ ID NO: 42 - DNA, 1416 bp, synthetic construct
  misc_feature 1..1416: note = Mouse NME8 variant2
  source 1..1416: mol_type = other DNA
atggcaagcaaaaagcgtgaagtccagctacagtcagtcgtcaatagtcagaacttgtgggatgagatgttgctgaacaaaggcttaacagtgattgatgtttaccaagcctggtgtggaccttgcaaagccgtgcaaagtttattcagaaaactaaaaaatgaactgaacgaagatgagattcttcacttcgtcgttgctgaagctgacaacattgtgactctccagccatttagagataaatgtgagcccgtgtttctctttagtcttaatggtaaaatcattgcaaagattcagggtgcaaatgctccacttatcaatagaaaagtcattaccttgatagatgaagagaggaaaattgtagcaggtgaaatggatcgtcctcagtatgttgaaattccactagtagatgcaatcgatgaagaatatggggaagtacagtatgaaagtgctgcggaagtttacaatatggcaattatcaaacctgatgctgtactcatgagaaaaaatatagaagttagggaaaaaatagccaaagaaggatttgttatagaaatacaagaaaacctgattctccctgaagaggtagtgagggaattctacactcatatagcagaccagcctgactttgaagagtttgtcgtttctatgacaaatggcctcagctgtgtgctcattgtatctcaagaagactccgaggttattcaggaagaaactctcccgcagactgatacagaagaagaacctggcgttttggaagagcctcacgttaggtttgcacctgtgatgataaagaagaaacgggacagtttgcaagagtatatggaccgacagcatatgtctgattactgcgatgtcgaggacgatgcggttaaggtctctaagctcattgacatattattccctgattttaaaactatgaaaagcacgaatgtacaaacgacgctagcattactgcatccagacatctgtgaggaagagaaagatgacgtgttgaacgttattcacaatgaagggttcaccatactgatgcagaggcaaatcgtattatcagaggaagaagcaagaacagtgtgcaagatccatgaaaacgaagagtattttgataatcttatagggcacatgaccagtaatcactcttatgtccttgctctacggagggaaaatggtgtggaatattggaaaacattaattgggccaaaaacgattgaggaagcttatgcatctcatccacagagtttatgtgtacagtttgcttcagggaattttcctaccaaccagttctacgggagcagttcaaaagcagcagctgagaaggaaatagcgcatttcttccctccccagagcacacttgcattgatcaagcctcatgtgacacacaaagaaagaattcacagaagctcaaggaggtaatga

SEQ ID NO: 43 - protein, 470 aa, synthetic construct
  REGION 1..470: note = Mouse NME8 variant2
MASKKREVQLQSVVNSQNLWDEMLLNKGLTVIDVYQAWCGPCKAVQSLFRKLKNELNEDEILHFVVAEADNIVTLQPFRDKCEPVFLFSLNGKIIAKIQGANAPLINRKVITLIDEERKIVAGEMDRPQYVEIPLVDAIDEEYGEVQYESAAEVYNMAIIKPDAVLMRKNIEVREKIAKEGFVIEIQENLILPEEVVREFYTHIADQPDFEEFVVSMTNGLSCVLIVSQEDSEVIQEETLPQTDTEEEPGVLEEPHVRFAPVMIKKKRDSLQEYMDRQHMSDYCDVEDDAVKVSKLIDILFPDFKTMKSTNVQTTLALLHPDICEEEKDDVLNVIHNEGFTILMQRQIVLSEEEARTVCKIHENEEYFDNLIGHMTSNHSYVLALRRENGVEYWKTLIGPKTIEEAYASHPQSLCVQFASGNFPTNQFYGSSSKAAAEKEIAHFFPPQSTLALIKPHVTHKERIHRSSRR

SEQ ID NO: 44 - DNA, 1767 bp, synthetic construct
  misc_feature 1..1767: note = Human NME8
  source 1..1767: mol_type = other DNA
atggcaagcaaaaaacgagaagtccagttacagacagtcatcaataatcaaagcctgtgggatgagatgttgcagaacaaaggcttaacagtgattgatgtttaccaagcctggtgtggaccttgcagagcaatgcaacctttattcagaaaattgaaaaatgaactgaacgaagacgaaattctgcattttgctgtcgcagaagctgacaacattgtgactttgcagccatttagagataaatgtgaacctgtttttctctttagtgttaatggcaaaattatcgaaaagattcagggtgcaaatgcaccgcttgttaataaaaaagttattaatttgatcgatgaggagagaaaaattgcagcaggtgaaatggctcgacctcagtatcctgaaattccattagtagactcagattcagaagttagtgaagaatcaccatgtgaaagtgttcaggaattatacagtattgctattatcaaaccggatgctgtgattagtaaaaaagttctagaaattaaaagaaaaattaccaaagctggatttattatagaagcagagcataagacagtgctcactgaagaacaagttgtcaacttctatagtcgaatagcagaccagcgtgacttcgaagagtttgtctcttttatgacaagtggcttaagctatattctagttgtatctcaaggaagtaaacacaatcctccctctgaagaaaccgaaccacagactgacaccgaacctaacgaacgatctgaggatcaacctgaggtcgaagcccaggttacacctggaatgatgaagaacaaacaagacagtttacaagaatatctggaaagacaacatttagctcagctctgtgacattgaagaggatgcagctaatgttgctaagttcatggatgctttcttccccgattttaaaaaaatgaaaagcatgaaattagaaaagacattggcattacttcgaccaaatctctttcatgaaaggaaagatgatgttttgcgtattattaaagatgaagacttcaaaatactggagcaaagacaagtagtattatcggaaaaagaagcacaagcactgtgcaaggaatatgaaaatgaagactattttaataaacttatagaaaacatgaccagtggtccatctctagcccttgttttattgagagacaatggcttgcaatactggaaacaattactgggaccaagaactgttgaagaagccattgaatattttccagagagtttatgtgcacagtttgcgatggacagtttgccggtcaaccagttgtatggcagcgattcattagaaaccgctgaaagggaaatacagcatttctttcctcttcaaagcactttaggcttgattaaacctcatgcaacaagtgaacaaagagagcagatcctgaagatagttaaggaggctggatttgatctgacacaggtgaagaaaatgttcctaactcctgagcaaacggagaaaatttatccaaaagtaacaggaaaagacttttataaagatttattggaaatgttatctgtgggtccatctatggtcatgattctgaccaagtggaatgctgttgcagaatggagacgattgatgggcccaacagacccagaagaagcaaaattactttcccctgactccatccgagcccagtttggaataagtaaattgaaaaacattgtccatggagcatctaacgcctatgaagcaaaagaggttgttaatagactctttgaggatcctgaggaaaactaa

SEQ ID NO: 45 - protein, 588 aa, synthetic construct
  REGION 1..588: note = Human NME8
MASKKREVQLQTVINNQSLWDEMLQNKGLTVIDVYQAWCGPCRAMQPLFRKLKNELNEDEILHFAVAEADNIVTLQPFRDKCEPVFLFSVNGKIIEKIQGANAPLVNKKVINLIDEERKIAAGEMARPQYPEIPLVDSDSEVSEESPCESVQELYSIAIIKPDAVISKKVLEIKRKITKAGFIIEAEHKTVLTEEQVVNFYSRIADQRDFEEFVSFMTSGLSYILVVSQGSKHNPPSEETEPQTDTEPNERSEDQPEVEAQVTPGMMKNKQDSLQEYLERQHLAQLCDIEEDAANVAKFMDAFFPDFKKMKSMKLEKTLALLRPNLFHERKDDVLRIIKDEDFKILEQRQVVLSEKEAQALCKEYENEDYFNKLIENMTSGPSLALVLLRDNGLQYWKQLLGPRTVEEAIEYFPESLCAQFAMDSLPVNQLYGSDSLETAEREIQHFFPLQSTLGLIKPHATSEQREQILKIVKEAGFDLTQVKKMFLTPEQTEKIYPKVTGKDFYKDLLEMLSVGPSMVMILTKWNAVAEWRRLMGPTDPEEAKLLSPDSIRAQFGISKLKNIVHGASNAYEAKEVVNRLFEDPEEN

SEQ ID NO: 46 - DNA, 1458 bp, synthetic construct
  misc_feature 1..1458: note = NME8 E. coli optimized
  source 1..1458: mol_type = other DNA
atgctggtcaataaaaaagtcatcaacctgatcgacgaagaacgcaaaatcgccgctggtgaaatggcacgcccgcaatacccggaaatcccgctggttgatagcgactctgaagtttcagaagaatcgccgtgcgaatcagtgcaggaactgtattcgatcgcaattatcaaaccggatgctgtcatttccaaaaaagtgctggaaatcaaacgtaaaatcaccaaagcgggtttcattatcgaagccgaacataaaaccgtgctgacggaagaacaggtggttaatttttattcacgtatcgcggatcagcgcgactttgaagaatttgtttcgtttatgaccagcggcctgtcttacattctggtcgtgagtcagggttccaaacacaatccgccgagcgaagaaacggaaccgcagaccgatacggaaccgaacgaacgttctgaagaccagccggaagtggaagcacaagttaccccgggcatgatgaaaaataaacaggatagtctgcaagaatacctggaacgccagcatctggctcaactgtgtgatatcgaagaagacgcggccaacgtggcgaaattcatggatgcctttttcccggacttcaagaaaatgaaaagcatgaaactggaaaaaaccctggccctgctgcgtccgaacctgttccacgaacgtaaagatgacgttctgcgcatcatcaaagatgaagacttcaaaatcctggaacagcgccaagttgtcctgtctgaaaaagaagcacaggctctgtgcaaagaatacgaaaacgaagattacttcaacaaactgatcgaaaacatgacctcaggtccgtcgctggcactggttctgctgcgtgataatggcctgcagtattggaaacaactgctgggtccgcgcacggtcgaagaagccattgaatacttcccggaaagcctgtgtgcacagtttgctatggattctctgccggtgaaccaactgtatggcagtgactccctggaaaccgcggaacgtgaaatccagcatttctttccgctgcaaagtaccctgggtctgattaaaccgcacgcgacgtccgaacagcgcgaacaaattctgaaaatcgtcaaagaagccggcttcgatctgacccaggtgaagaaaatgtttctgaccccggaacaaacggaaaaaatctatccgaaagtcacgggcaaagatttctacaaagacctgctggaaatgctgagtgttggtccgtccatggtcatgattctgaccaaatggaatgcggttgcagaatggcgtcgcctgatgggtccgacggatccggaagaagcaaaactgctgagcccggactctattcgcgctcagtttggcatcagcaaactgaaaaacattgttcatggtgcgtccaatgcgtatgaagcgaaagaagttgtgaaccgcctgtttgaagacccggaagaaaattaa

SEQ ID NO: 47 - protein, 485 aa, synthetic construct
  REGION 1..485: note = NME8 E. coli optimized
MLVNKKVINLIDEERKIAAGEMARPQYPEIPLVDSDSEVSEESPCESVQELYSIAIIKPDAVISKKVLEIKRKITKAGFIIEAEHKTVLTEEQVVNFYSRIADQRDFEEFVSFMTSGLSYILVVSQGSKHNPPSEETEPQTDTEPNERSEDQPEVEAQVTPGMMKNKQDSLQEYLERQHLAQLCDIEEDAANVAKFMDAFFPDFKKMKSMKLEKTLALLRPNLFHERKDDVLRIIKDEDFKILEQRQVVLSEKEAQALCKEYENEDYFNKLIENMTSGPSLALVLLRDNGLQYWKQLLGPRTVEEAIEYFPESLCAQFAMDSLPVNQLYGSDSLETAEREIQHFFPLQSTLGLIKPHATSEQREQILKIVKEAGFDLTQVKKMFLTPEQTEKIYPKVTGKDFYKDLLEMLSVGPSMVMILTKWNAVAEWRRLMGPTDPEEAKLLSPDSIRAQFGISKLKNIVHGASNAYEAKEVVNRLFEDPEEN

SEQ ID NO: 48 - DNA, 1062 bp, synthetic construct
  misc_feature 1..1062: note = NME8 1-2 E. coli optimized
  source 1..1062: mol_type = other DNA
atgctggtcaataaaaaagtcatcaacctgatcgacgaagaacgcaaaatcgccgctggtgaaatggcacgcccgcaatacccggaaatcccgctggttgatagcgactctgaagtttcagaagaatcgccgtgcgaatcagtgcaggaactgtattcgatcgcaattatcaaaccggatgctgtcatttccaaaaaagtgctggaaatcaaacgtaaaatcaccaaagcgggtttcattatcgaagccgaacataaaaccgtgctgacggaagaacaggtggttaatttttattcacgtatcgcggatcagcgcgactttgaagaatttgtttcgtttatgaccagcggcctgtcttacattctggtcgtgagtcagggttccaaacacaatccgccgagcgaagaaacggaaccgcagaccgatacggaaccgaacgaacgttctgaagaccagccggaagtggaagcacaagttaccccgggcatgatgaaaaataaacaggatagtctgcaagaatacctggaacgccagcatctggctcaactgtgtgatatcgaagaagacgcggccaacgtggcgaaattcatggatgcctttttcccggacttcaagaaaatgaaaagcatgaaactggaaaaaaccctggccctgctgcgtccgaacctgttccacgaacgtaaagatgacgttctgcgcatcatcaaagatgaagacttcaaaatcctggaacagcgccaagttgtcctgtctgaaaaagaagcacaggctctgtgcaaagaatacgaaaacgaagattacttcaacaaactgatcgaaaacatgacctcaggtccgtcgctggcactggttctgctgcgtgataatggcctgcagtattggaaacaactgctgggtccgcgcacggtcgaagaagccattgaatacttcccggaaagcctgtgtgcacagtttgctatggattctctgccggtgaaccaactgtatggcagtgactccctggaaaccgcggaacgtgaaatccagcatttctttctcgagcaccaccaccaccaccactga

SEQ ID NO: 49 - protein, 353 aa, synthetic construct
  REGION 1..353: note = NME8 1-2 E. coli optimized
MLVNKKVINLIDEERKIAAGEMARPQYPEIPLVDSDSEVSEESPCESVQELYSIAIIKPDAVISKKVLEIKRKITKAGFIIEAEHKTVLTEEQVVNFYSRIADQRDFEEFVSFMTSGLSYILVVSQGSKHNPPSEETEPQTDTEPNERSEDQPEVEAQVTPGMMKNKQDSLQEYLERQHLAQLCDIEEDAANVAKFMDAFFPDFKKMKSMKLEKTLALLRPNLFHERKDDVLRIIKDEDFKILEQRQVVLSEKEAQALCKEYENEDYFNKLIENMTSGPSLALVLLRDNGLQYWKQLLGPRTVEEAIEYFPESLCAQFAMDSLPVNQLYGSDSLETAEREIQHFFLEHHHHHH

SEQ ID NO: 50 - DNA, 852 bp, synthetic construct
  misc_feature 1..852: note = NME8 2-3 E coli optimized
  source 1..852: mol_type = other DNA
atgctggaaaaaaccctggccctgctgcgtccgaacctgttccacgaacgtaaagatgacgttctgcgcatcatcaaagatgaagacttcaaaatcctggaacagcgccaagttgtcctgtctgaaaaagaagcacaggctctgtgcaaagaatacgaaaacgaagattacttcaacaaactgatcgaaaacatgacctcaggtccgtcgctggcactggttctgctgcgtgataatggcctgcagtattggaaacaactgctgggtccgcgcacggtcgaagaagccattgaatacttcccggaaagcctgtgtgcacagtttgctatggattctctgccggtgaaccaactgtatggcagtgactccctggaaaccgcggaacgtgaaatccagcatttctttccgctgcaaagtaccctgggtctgattaaaccgcacgcgacgtccgaacagcgcgaacaaattctgaaaatcgtcaaagaagccggcttcgatctgacccaggtgaagaaaatgtttctgaccccggaacaaacggaaaaaatctatccgaaagtcacgggcaaagatttctacaaagacctgctggaaatgctgagtgttggtccgtccatggtcatgattctgaccaaatggaatgcggttgcagaatggcgtcgcctgatgggtccgacggatccggaagaagcaaaactgctgagcccggactctattcgcgctcagtttggcatcagcaaactgaaaaacattgttcatggtgcgtccaatgcgtatgaagcgaaagaagttgtgaaccgcctgtttgaagacccggaagaaaatctcgagcaccaccaccaccaccactga

SEQ ID NO: 51 - protein, 283 aa, synthetic construct
  REGION 1..283: note = NME8 2-3 E coli optimized
MLEKTLALLRPNLFHERKDDVLRIIKDEDFKILEQRQVVLSEKEAQALCKEYENEDYFNKLIENMTSGPSLALVLLRDNGLQYWKQLLGPRTVEEAIEYFPESLCAQFAMDSLPVNQLYGSDSLETAEREIQHFFPLQSTLGLIKPHATSEQREQILKIVKEAGFDLTQVKKMFLTPEQTEKIYPKVTGKDFYKDLLEMLSVGPSMVMILTKWNAVAEWRRLMGPTDPEEAKLLSPDSIRAQFGISKLKNIVHGASNAYEAKEVVNRLFEDPEENLEHHHHHH